European Patent Specification EP 4 208 718 B1, published April 16, 2025. Title: PREDICTING CANCER RELAPSE AND TREATMENT OF CANCER DISEASES. Applicant: Johansson Swartling, Fredrik Hutter, Sonja. The sequence listing filed with the application follows.

SEQUENCE LISTING (14 sequences)

SEQ ID NO: 1 - DNA, 4000 bp, Homo sapiens
  misc_feature (2501)..(2501): Transcription start site
cagtccccaaattctgcgcagaatagaacggctggcatctcaagtgctcttttttcacccggatctctacagacacaagttccctcactgagctgcgcagaggtggatccgcacaggagggaatatcgcgtaggaattcctgcaaatataaatctcagcagcaaagcagtccagattgactggaacacaccacccccagccaccaccatccaagttttccctggttctcggagttggaaacagtttctgggcttttggcgccccctctggatacagatgaaaactgcagtccatttttaagtcgcctgttcataagttttcaggaagatgtaaaattcaaaaatgcttgcatcaaatcaacgggaaatgtataaatccccgtcgtttatgatgtaaaactctacatattagtatcttattgcataattgcattaaaagtatatttatacatatacgtatatatcttgacatatatttagtgaaatattccaaaatatcttaaagtcatagccctcttcactgactttattccagcaaacatggtaattacaatatcatacaactaagtacagacgacctggctaaaatgtctgcccgatggtctccgagtctcctgaatcaggtgtctgagaattacacagttatactgtacacacaatgcccttctacccgggacacagaaataggtccacactacgcggacttttttctcctaggaaaggacgatgctgttcttacactttctgaaagtaatcacagagccctggatacgaagctattgtatgcaaatctcttaaatttgtaaacgagctatagggcaccagaaacatcccatttgaagaagttacattcgttaaaaaaaaaatgctgttgaacaaggctgtaacttactaccttatgaagagttccatttcctataagaaatgtcgggcttcttccgaagacaacgagagaaaacaagattttaagaaattctcccggaaggacattgatttggatcttgtgatagtgtcctcacttcgcaaattagaaagggaaaaaaaaactagtttttattatgatgtgggccgattcaccacaacaataatttaattgaggcgaatttttgcaagagcccaaaagggtggggggggggggggagtttaaaattaagagtttcccaatgctgtgcgtttatttgggattctgaaagcacagaacccgcaagcgaccaagacttttcttctatcccagagcagatagctccgcacttacccaacctggctctaagcatttcgtgtaaacacaaaggttgtgctcaaatcacacttgaaatacatgagagacaccaccaatgcctcccccagaactcccaactacatgcaggtctgaaccgaccggactagagtcagaagcaccggcgcttcaccccttcaggtgtttcgtaaatgccagcaaaagcaggcaagcagcatgactccgccagagtggagcgttttgtctgcggtggtgcccatttgtttggtcttttacaaaccaagtgaccggcctgggcctcgcggcccgggacagccgcattggcaaacttctatctctcaaagccagagcagttagcaaactctcccccagacagggcgactcggctgacgtttttgacccggccaggaggcaaagaccaaaacgtcagagcagtagccctgttactgaggagcgtcggcagggtcgcgggtagagggggctggagaatgacttgtcagagctcaaggtcgatgtggcgcggggcggcctcgagagcgccgggctcctgcgtggccacggccgccgctgccaaccttcgcggggacttagctttgctttccattgactccctttgcaaaagcgcagcagaatcctgaccagccgcaccagccccggcgaacccgagcatgttaatctatttatatggattattacggaggaacagcgggcgttgagtcaccaaaacatttgcttcaaaagactatttctaagcacttttgcaggcaggcaggctcgctccaggcgcgtaaactcggctacgcattaagaagcggctgcttttcgaatactgcaaactccagctaagtccccggtgccgcggagagagcagtgaaaagaaatgtcggaggtgggggtagatcctagtctagacacacacacttgcgcgcacacacacacacacacacacaagattcgcgcggagaaggcactaaaattctggcattccgagagtacgacaaacttacacacttggaagtcccgggtcccccgccttccccgcagcaccccccgcccccccaccctaccgtccgccctttggctgcgatcccctcccctctcctcccctcccgcctcgtcacccagcccagtgccacaatcctcctccctccccaaaatcgggtccaatcagctgcctgccaaccctgggactgctgtgctgtgattggcgggtggctctaaggtgaggcggagtatttattaaagagaccctgggctgggagttggagagccgaaagcggagctcgaaactgactggaaacttcagtggcgcggagactcgccagtttcaaccccggaaacttttctttgcaggaggagaagagaaggggtgcaagcgcccccacttttgctctttttcctcccctcctcctcctctccaattcgcctccccccacttggagcgggcagctgtgaactggccaccccgcgccttcctaagtgctcgccgcggtagccggccgacgcgccagcttccccgggagccgcttgctccgcatccgggcagccgaggggagaggagcccgcgcctcgagtccccgagccgccgcggcttctcgcctttcccggccaccagccccctgccccgggcccgcgtatgaatctcctggaccccttcatgaagatgaccgacgagcaggagaagggcctgtccggcgcccccagccccaccatgtccgaggactccgcgggctcgccctgcccgtcgggctccggctcggacaccgagaacacgcggccccaggagaacacgttccccaagggcgagcccgatctgaagaaggagagcgaggaggacaagttccccgtgtgcatccgcgaggcggtcagccaggtgctcaaaggctacgactggacgctggtgcccatgccggtgcgcgtcaacggctccagcaagaacaagccgcacgtcaagcggcccatgaacgccttcatggtgtgggcgcaggcggcgcgcaggaagctcgcggaccagtacccgcacttgcacaacgccgagctcagcaagacgctgggcaagctctggaggtaggacccggcgggggcggcgcggcagggtgggcatcgcggcggctgggggcgctggtcagggctgatttgccccgccccgcctcccatcgcccgggagttgccgttccgggagccggcgggatggggttgggagtgggaatggggtgtaactgtggctcagagtttgacaaagttcttgggctgctcgcggggacgcggaggaggggggtggtaagtggaagaggtgagggaggtagctggaggatggacgaagactggtgggagacggaaggagggggctgccagcctgctctccagtcgcctggaagctcaatcggggcggggaagtgaaacttgcctccctcctacccggcctcttaaaactgcactctctcgtgcagccccactgtccacggagatggggcaagggagaaaccgaggttggaggagacccttggcaggaactgggaggcgggaggagggaggctactggaaataggtgggagtgtatggtggggggtgagaattggggaccttcttgcagcttaagtaatttgggggaaagttttcaaagggggttggggttgggggcggtaagtcgagcagcaaaggcgtttagggggcagcaccgggagtcgttttcatctccagcgtttccaaaatagaaatagaaggggaggggagggagggggcggggagtgaccgctcaggtcag

SEQ ID NO: 2 - DNA, 1600 bp, Homo sapiens
  misc_feature (1351)..(1351): Transcription starting site
aagagtttcccaatgctgtgcgtttatttgggattctgaaagcacagaacccgcaagcgaccaagacttttcttctatcccagagcagatagctccgcacttacccaacctggctctaagcatttcgtgtaaacacaaaggttgtgctcaaatcacacttgaaatacatgagagacaccaccaatgcctcccccagaactcccaactacatgcaggtctgaaccgaccggactagagtcagaagcaccggcgcttcaccccttcaggtgtttcgtaaatgccagcaaaagcaggcaagcagcatgactccgccagagtggagcgttttgtctgcggtggtgcccatttgtttggtcttttacaaaccaagtgaccggcctgggcctcgcggcccgggacagccgcattggcaaacttctatctctcaaagccagagcagttagcaaactctcccccagacagggcgactcggctgacgtttttgacccggccaggaggcaaagaccaaaacgtcagagcagtagccctgttactgaggagcgtcggcagggtcgcgggtagagggggctggagaatgacttgtcagagctcaaggtcgatgtggcgcggggcggcctcgagagcgccgggctcctgcgtggccacggccgccgctgccaaccttcgcggggacttagctttgctttccattgactccctttgcaaaagcgcagcagaatcctgaccagccgcaccagccccggcgaacccgagcatgttaatctatttatatggattattacggaggaacagcgggcgttgagtcaccaaaacatttgcttcaaaagactatttctaagcacttttgcaggcaggcaggctcgctccaggcgcgtaaactcggctacgcattaagaagcggctgcttttcgaatactgcaaactccagctaagtccccggtgccgcggagagagcagtgaaaagaaatgtcggaggtgggggtagatcctagtctagacacacacacttgcgcgcacacacacacacacacacacaagattcgcgcggagaaggcactaaaattctggcattccgagagtacgacaaacttacacacttggaagtcccgggtcccccgccttccccgcagcaccccccgcccccccaccctaccgtccgccctttggctgcgatcccctcccctctcctcccctcccgcctcgtcacccagcccagtgccacaatcctcctccctccccaaaatcgggtccaatcagctgcctgccaaccctgggactgctgtgctgtgattggcgggtggctctaaggtgaggcggagtatttattaaagagaccctgggctgggagttggagagccgaaagcggagctcgaaactgactggaaacttcagtggcgcggagactcgccagtttcaaccccggaaacttttctttgcaggaggagaagagaaggggtgcaagcgcccccacttttgctctttttcctcccctcctcctcctctccaattcgcctccccccacttggagcgggcagctgtgaactggccaccccgcgccttcctaagtgctcgccgcggtagccggccgacgcgccagctt

SEQ ID NO: 3 - DNA, 323 bp, Homo sapiens
  misc_feature (257)..(257): Transcription start site
cacttggaagtcccgggtcccccgccttccccgcagcaccccccgcccccccaccctaccgtccgccctttggctgcgatcccctcccctctcctcccctcccgcctcgtcacccagcccagtgccacaatcctcctccctccccaaaatcgggtccaatcagctgcctgccaaccctgggactgctgtgctgtgattggcgggtggctctaaggtgaggcggagtatttattaaagagaccctgggctgggagttggagagccgaaagcggagctcgaaactgactggaaacttcagtggcgcggagactcgccagtttcaa

SEQ ID NO: 4 - DNA, 1101 bp, Homo sapiens
  misc_feature (1035)..(1035): Transcription start site
gtggagcgttttgtctgcggtggtgcccatttgtttggtcttttacaaaccaagtgaccggcctgggcctcgcggcccgggacagccgcattggcaaacttctatctctcaaagccagagcagttagcaaactctcccccagacagggcgactcggctgacgtttttgacccggccaggaggcaaagaccaaaacgtcagagcagtagccctgttactgaggagcgtcggcagggtcgcgggtagagggggctggagaatgacttgtcagagctcaaggtcgatgtggcgcggggcggcctcgagagcgccgggctcctgcgtggccacggccgccgctgccaaccttcgcggggacttagctttgctttccattgactccctttgcaaaagcgcagcagaatcctgaccagccgcaccagccccggcgaacccgagcatgttaatctatttatatggattattacggaggaacagcgggcgttgagtcaccaaaacatttgcttcaaaagactatttctaagcacttttgcaggcaggcaggctcgctccaggcgcgtaaactcggctacgcattaagaagcggctgcttttcgaatactgcaaactccagctaagtccccggtgccgcggagagagcagtgaaaagaaatgtcggaggtgggggtagatcctagtctagacacacacacttgcgcgcacacacacacacacacacacaagattcgcgcggagaaggcactaaaattctggcattccgagagtacgacaaacttacacacttggaagtcccgggtcccccgccttccccgcagcaccccccgcccccccaccctaccgtccgccctttggctgcgatcccctcccctctcctcccctcccgcctcgtcacccagcccagtgccacaatcctcctccctccccaaaatcgggtccaatcagctgcctgccaaccctgggactgctgtgctgtgattggcgggtggctctaaggtgaggcggagtatttattaaagagaccctgggctgggagttggagagccgaaagcggagctcgaaactgactggaaacttcagtggcgcggagactcgccagtttcaa

SEQ ID NO: 5 - RNA, 36 nt, Artificial Sequence
  crRNA targeting SOX9
guucaccgauguccacgucgguuuuagagcuaugcu

SEQ ID NO: 6 - RNA, 36 nt, Artificial Sequence
  crRNA targeting SOX9
accaugucggaggacucggcguuuuagagcuaugcu

SEQ ID NO: 7 - RNA, 36 nt, Artificial Sequence
  crRNA targeting SOX9
gaagggcuacgacuggacgcguuuuagagcuaugcu

SEQ ID NO: 8 - DNA, 21 bp, Artificial Sequence
  PCR forward primer
ccggccccaggagaacacctt

SEQ ID NO: 9 - DNA, 20 bp, Artificial Sequence
  PCR reverse primer
gtgagtgcagcccgcgtccc

SEQ ID NO: 10 - DNA, 23 bp, Artificial Sequence
  SOX9 forward primer
tcaacggctccagcaagaacaag

SEQ ID NO: 11 - DNA, 24 bp, Artificial Sequence
  SOX9 reverse primer
acttgtaatccgggtggtccttct

SEQ ID NO: 12 - DNA, 49 bp, Homo sapiens
ctgtgaatcgggctctgtgtgcgctcgagaaaagccccattcatgagag

SEQ ID NO: 13 - DNA, 196 bp, Homo sapiens
ctgtgaatcgggctctgtgtgcgctcgagaaaagccccattcatgagagctgtgaatcgggctctgtgtgcgctcgagaaaagccccattcatgagagctgtgaatcgggctctgtgtgcgctcgagaaaagccccattcatgagagctgtgaatcgggctctgtgtgcgctcgagaaaagccccattcatgagag

SEQ ID NO: 14 - DNA, 198 bp, Homo sapiens
ctgtgaatcgggctctgtgtgcgctcgagaaaagccccattcatgagagctgtgaatcgggctctgtgtgcgctcgagaaaagccccattcatgagagctgtgaatcgggctctgtgtgcgctcgagaaaagccccattcatgagagctgtgaatcgggctctgtgtgcgctcgagaaaagccccattcatgagagct